European Patent Application EP 4 556 003 A1, published May 21, 2025. Title: ANTI-OBESITY AND ANTI-DIABETIC ACTIVITY OF BROMINATED DITERPENES FROM RED ALGAE OF THE GENUS LAURENCIA AND APPLICATIONS THEREOF. Applicant: NATIONAL AND KAPODISTRIAN UNIVERSITY OF ATHENS. Application EP. The sequence listing filed with the application follows.

SEQUENCE LISTING (28 sequences)

SEQ ID NO: 1 - DNA, 20 bp, artificial sequence
  source 1..20: mol_type = genomic DNA
gccccattccctggttcatt

SEQ ID NO: 2 - DNA, 20 bp, artificial sequence
  source 1..20: mol_type = genomic DNA
gacccatagcatccgcaaca

SEQ ID NO: 3 - DNA, 20 bp, artificial sequence
  source 1..20: mol_type = genomic DNA
ttcacacacgcagtcggtat

SEQ ID NO: 4 - DNA, 20 bp, artificial sequence
  source 1..20: mol_type = genomic DNA
tcattggctatctgcagcac

SEQ ID NO: 5 - DNA, 22 bp, artificial sequence
  source 1..22: mol_type = genomic DNA
aaaggagatgcaggtcttcttg

SEQ ID NO: 6 - DNA, 21 bp, artificial sequence
  source 1..21: mol_type = genomic DNA
ctgagcgatacacataagcgg

SEQ ID NO: 7 - DNA, 20 bp, artificial sequence
  source 1..20: mol_type = genomic DNA
aagtgtgtaactgcccctgg

SEQ ID NO: 8 - DNA, 20 bp, artificial sequence
  source 1..20: mol_type = genomic DNA
tgcaagcccgaacgtctatt

SEQ ID NO: 9 - DNA, 22 bp, artificial sequence
  source 1..22: mol_type = genomic DNA
gctcctcctcgaaggtttacaa

SEQ ID NO: 10 - DNA, 22 bp, artificial sequence
  source 1..22: mol_type = genomic DNA
aatccccatttacgctgatgat

SEQ ID NO: 11 - DNA, 20 bp, artificial sequence
  source 1..20: mol_type = genomic DNA
gctggcctccttgatgaata

SEQ ID NO: 12 - DNA, 20 bp, artificial sequence
  source 1..20: mol_type = genomic DNA
ttgggctccataaagtcacc

SEQ ID NO: 13 - DNA, 20 bp, artificial sequence
  source 1..20: mol_type = genomic DNA
gactcggctactgacacgac

SEQ ID NO: 14 - DNA, 20 bp, artificial sequence
  source 1..20: mol_type = genomic DNA
cgagttgagctgggttaggg

SEQ ID NO: 15 - DNA, 20 bp, artificial sequence
  source 1..20: mol_type = genomic DNA
ctgcaccaccaactgcttag

SEQ ID NO: 16 - DNA, 18 bp, artificial sequence
  source 1..18: mol_type = genomic DNA
gggccatccacagtcttc

SEQ ID NO: 17 - DNA, 20 bp, artificial sequence
  source 1..20: mol_type = genomic DNA
tcaccgaccctcgttgccca

SEQ ID NO: 18 - DNA, 20 bp, artificial sequence
  source 1..20: mol_type = genomic DNA
tgcttcacagcctcacgccg

SEQ ID NO: 19 - DNA, 20 bp, artificial sequence
  source 1..20: mol_type = genomic DNA
gagaaccgtggactggacaa

SEQ ID NO: 20 - DNA, 20 bp, artificial sequence
  source 1..20: mol_type = genomic DNA
gacacgtcacatttcggagc

SEQ ID NO: 21 - DNA, 24 bp, artificial sequence
  source 1..24: mol_type = genomic DNA
gcgctgtcatcgatttctcccctg

SEQ ID NO: 22 - DNA, 25 bp, artificial sequence
  source 1..25: mol_type = genomic DNA
ggccttgtagacaccttggtcttgg

SEQ ID NO: 23 - DNA, 25 bp, artificial sequence
  source 1..25: mol_type = genomic DNA
acctgctgggaaggaagaaaaggcc

SEQ ID NO: 24 - DNA, 24 bp, artificial sequence
  source 1..24: mol_type = genomic DNA
aagccactgccgtgttcacagtac

SEQ ID NO: 25 - DNA, 22 bp, artificial sequence
  source 1..22: mol_type = genomic DNA
acagcaagttccatcgtgtcat

SEQ ID NO: 26 - DNA, 22 bp, artificial sequence
  source 1..22: mol_type = genomic DNA
gaagaactgtgagccattggtg

SEQ ID NO: 27 - DNA, 23 bp, artificial sequence
  source 1..23: mol_type = genomic DNA
cattgctgacaggatgcagaagg

SEQ ID NO: 28 - DNA, 22 bp, artificial sequence
  source 1..22: mol_type = genomic DNA
tgctggaaggtggacagtgagg